European Patent Application EP 4 640 829 A1, published October 29, 2025. Title: MUTATED LIPASE. Applicant: WILMAR (SHANGHAI) BIOTECHNOLOGY RESEARCH & DEVELOPMENT CENTER CO., LTD. The sequence listing filed with the application follows.

SEQUENCE LISTING (12 sequences)

SEQ ID NO: 1 - protein, 269 aa, synthetic construct
DVSQDLFDQFNLFAQYSAAAYCAKNNDAPAGAIVTCRGSICPEVEKADATFLYSFEDSGVGDVTGFLALDNTNRLIVLSFRGSRSLENWIGNINMDLKGIDDICSGCKGHDGFTSSWRSVANTLTQQVQNAVREHPDYRVVFTGHSLGGALATVAGASLRGNGYDIDVFSYGAPRVGNRAFAEFLTAQTGGTLYRITHTNDIVPRLPPRELGYSHSSPEYWITSGTLVPVRRRDIVKVEGIDSTDGNNQPNTPDIAAHFWYFGSIGTCL

SEQ ID NO: 2 - protein, 269 aa, synthetic construct
DVSQDLFDQFNLFAQYSAAAYCAKNNRAPAGAIVTCRASICPEVEKADATFLYSFEDSGVGDVTGFLALDNTNRLIVLSFRGSRSLENWIGNINMELKGIDDICSGCKGHAGFTSSWRSVANTLTQQVQNAVREHPDYRVVFTGHSLGGALATVAGASLRGNKYDIDVFSYGAPRVGNRAFAEFLTAQTGGTLYRITHTNDIVPRLPPRELGYSHSSPEYWITSGTLVPVRRRDIVKVEGIDSTDGNNQPNTPSITAHFWYFGSIGTCL

SEQ ID NO: 3 - DNA, 1077 bp, synthetic construct
  source 1..1077: mol_type = other DNA
atgagatttccttcaatttttactgcagttttattcgcagcatcctccgcattagctgctccagtcaacactacaacagaagatgaaacggcacaaattccggctgaagctgtcatcggttactcagatttagaaggggatttcgatgttgctgttttgccattttccaacagcacaaataacgggttattgtttataaatactactattgccagcattgctgctaaagaagaaggggtatctcttgagaaaagagaggctgaagctgatgtttctcaagatttgtttgatcaatttaatttgtttgctcaatattctgctgcagcttattgtgctaaaaataatagggctcctgctggtgctattgttacttgtagagcttctatttgtcctgaagttgaaaaagctgatgctacttttttgtattcttttgaagattctggtgttggtgatgttactggttttttggctttggataatactaatagattgattgttttgtcttttagaggttctaggtcattagaaaattggattggtaatattaacatggaattaaaaggtattgatgatatttgttctggttgtaaaggtcatgctggttttacttcttcttggaggtctgttgctaatactttgactcaacaagttcaaaatgctgttagagaacatcctgattatagagttgtttttactggtcattctttgggtggtgctttggctactgttgctggtgcttctttgagaggtaataaatatgatattgatgttttttcttatggtgctccaagagttggtaatagagcttttgctgaatttttgactgctcaaactggtggtactttgtatagaattactcatactaatgatattgttccaagattgccaccaagagaattgggttattctcattcttctcctgaatattggattacttctggtactttggttcctgttagaaggagagatattgttaaagttgaaggtattgattctactgatggtaataatcaaccaaatactccatctattactgctcatttttggtattttggttctattggtacttgtttgtaa

SEQ ID NO: 4 - protein, 269 aa, synthetic construct
DVSQDLFDQFNLFAQYSAAAYCAKNNRAPAGAIVTCRASICPEVEKADATFLYSFEDSGVGDVTGFLALDNTNRLIVLSFRGSRSIENWIGNLNFELKGIDDICSGCKGHAGFTSSWRSVANTLTQQVQNAVREHPDYRVVFTGHSLGGALATVAGASLRGNKYDIDVFSYGAPRVGNRAFAEFLTAQTGGTLYRITHTNDIVPRLPPRELGYSHSSPEYWITSGTLVPVRRRDIVKVEGIDSTDGNNQPNTPSITAHFWYFGSIGTCL

SEQ ID NO: 5 - DNA, 1077 bp, synthetic construct
  source 1..1077: mol_type = other DNA
atgagatttccttcaatttttactgcagttttattcgcagcatcctccgcattagctgctccagtcaacactacaacagaagatgaaacggcacaaattccggctgaagctgtcatcggttactcagatttagaaggggatttcgatgttgctgttttgccattttccaacagcacaaataacgggttattgtttataaatactactattgccagcattgctgctaaagaagaaggggtatctcttgagaaaagagaggctgaagctgatgtttctcaagatttgtttgatcaatttaatttgtttgctcaatattctgctgcagcttattgtgctaaaaataatagggctcctgctggtgctattgttacttgtagagcttctatttgtcctgaagttgaaaaagctgatgctacttttttgtattcttttgaagattctggtgttggtgatgttactggtttcttagcattggataatactaatagattgattgttttgtcattcagaggatctaggtctattgaaaattggatcggtaatttgaactttgaattgaaaggtattgatgatatttgttctggttgtaaaggtcatgctggttttacttcttcttggaggtctgttgctaatactttgactcaacaagttcaaaatgctgttagagaacatcctgattatagagttgtttttactggtcattctttgggtggtgctttggctactgttgctggtgcttctttgagaggtaataaatatgatattgatgttttttcttatggtgctccaagagttggtaatagagcttttgctgaatttttgactgctcaaactggtggtactttgtatagaattactcatactaatgatattgttccaagattgccaccaagagaattgggttattctcattcttctcctgaatattggattacttctggtactttggttcctgttagaaggagagatattgttaaagttgaaggtattgattctactgatggtaataatcaaccaaatactccatctattactgctcatttttggtattttggttctattggtacttgtttgtaa

SEQ ID NO: 6 - protein, 269 aa, synthetic construct
DVSQDLFDQFNLFAQYSAAAYCAKNNRAPAGAIVTCRASICPEVEKADATFLYSFEDSGVGDVTGFLALDNTNRLIVLSFRGSRSIENWIGNLNFELKGIDDICSGCKGHAGFTSSWRSVANTLTQQVQNAVREHPDYRVVFTGHSLGGALATVAGASLRGNKYDIDVFSYGAPRVGNRAFAEFLTAQTGGTLYRITHTNDIVPRLPPREFGYSHSSPEYWITSGTLVPVRRRDIVKVEGIDSTDGNNQPNTPSITAHFWYFGSIGTCL

SEQ ID NO: 7 - DNA, 1077 bp, synthetic construct
  source 1..1077: mol_type = other DNA
atgagatttccttcaatttttactgcagttttattcgcagcatcctccgcattagctgctccagtcaacactacaacagaagatgaaacggcacaaattccggctgaagctgtcatcggttactcagatttagaaggggatttcgatgttgctgttttgccattttccaacagcacaaataacgggttattgtttataaatactactattgccagcattgctgctaaagaagaaggggtatctcttgagaaaagagaggctgaagctgatgtttctcaagatttgtttgatcaatttaatttgtttgctcaatattctgctgcagcttattgtgctaaaaataatagggctcctgctggtgctattgttacttgtagagcttctatttgtcctgaagttgaaaaagctgatgctacttttttgtattcttttgaagattctggtgttggtgatgttactggtttcttagcattggataatactaatagattgattgttttgtcattcagaggatctaggtctattgaaaattggatcggtaatttgaactttgaattgaaaggtattgatgatatttgttctggttgtaaaggtcatgctggttttacttcttcttggaggtctgttgctaatactttgactcaacaagttcaaaatgctgttagagaacatcctgattatagagttgtttttactggtcattctttgggtggtgctttggctactgttgctggtgcttctttgagaggtaataaatatgatattgatgttttttcttatggtgctccaagagttggtaatagagcttttgctgaatttttgactgctcaaactggtggtactttgtatagaattactcatactaatgatattgttccaagattgccaccaagagaatttggttattctcattcttctcctgaatattggattacttctggtactttggttcctgttagaaggagagatattgttaaagttgaaggtattgattctactgatggtaataatcaaccaaatactccatctattactgctcatttttggtattttggttctattggtacttgtttgtaa

SEQ ID NO: 8 - protein, 269 aa, synthetic construct
DVSQDLFDQFNLFAQYSAAAYCAKNNRAPAGAIVTCRASICPEVEKADATFLYSFEDSGVGDVTGFLALDNTNRLIVLSFRGSRSIENWIGNLNWELKGIDDICSGCKGHAGFTSSWRSVANTLTQQVQNAVREHPDYRVVFTGHSLGGALATVAGASLRGNKYDIDVFSYGAPRVGNRAFAEFLTAQTGGTLYRITHTNDIVPRLPPREFGYSHSSPEYWITSGTLVPVRRRDIVKVEGIDSTDGNNQPNTPSITAHFWYFGSIGTCL

SEQ ID NO: 9 - DNA, 1077 bp, synthetic construct
  source 1..1077: mol_type = other DNA
atgagatttccttcaatttttactgcagttttattcgcagcatcctccgcattagctgctccagtcaacactacaacagaagatgaaacggcacaaattccggctgaagctgtcatcggttactcagatttagaaggggatttcgatgttgctgttttgccattttccaacagcacaaataacgggttattgtttataaatactactattgccagcattgctgctaaagaagaaggggtatctcttgagaaaagagaggctgaagctgatgtttctcaagatttgtttgatcaatttaatttgtttgctcaatattctgctgcagcttattgtgctaaaaataatagggctcctgctggtgctattgttacttgtagagcttctatttgtcctgaagttgaaaaagctgatgctacttttttgtattcttttgaagattctggtgttggtgatgttactggttttttggctttggataatactaatagattgattgttttgtcttttagaggatctaggtcaattgaaaactggattggtaatttgaattgggaattgaaaggtattgatgatatttgttctggttgtaaaggtcatgctggttttacttcttcttggaggtctgttgctaatactttgactcaacaagttcaaaatgctgttagagaacatcctgattatagagttgtttttactggtcattctttgggtggtgctttggctactgttgctggtgcttctttgagaggtaataaatatgatattgatgttttttcttatggtgctccaagagttggtaatagagcttttgctgaatttttgactgctcaaactggtggtactttgtatagaattactcatactaatgatattgttccaagattgccaccaagagaatttggttattctcattcttctcctgaatattggattacttctggtactttggttcctgttagaaggagagatattgttaaagttgaaggtattgattctactgatggtaataatcaaccaaatactccatctattactgctcatttttggtattttggttctattggtacttgtttgtaa

SEQ ID NO: 10 - protein, 269 aa, synthetic construct
DVSQDLFDQFNLFAQYSAAAYCAKNNRAPAGAIVTCRASICPEVEKADATFLYSFEDSGVGDVTGFLALDNTNRLIVLSFRGSRSIENWIGNLNYELKGIDDICSGCKGHAGFTSSWRSVANTLTQQVQNAVREHPDYRVVFTGHSLGGALATVAGASLRGNKYDIDVFSYGAPRVGNRAFAEFLTAQTGGTLYRITHTNDIVPRLPPREFGYSHSSPEYWITSGTLVPVRRRDIVKVEGIDSTDGNNQPNTPSITAHFWYFGSIGTCL

SEQ ID NO: 11 - DNA, 1077 bp, synthetic construct
  source 1..1077: mol_type = other DNA
atgagatttccttcaatttttactgcagttttattcgcagcatcctccgcattagctgctccagtcaacactacaacagaagatgaaacggcacaaattccggctgaagctgtcatcggttactcagatttagaaggggatttcgatgttgctgttttgccattttccaacagcacaaataacgggttattgtttataaatactactattgccagcattgctgctaaagaagaaggggtatctcttgagaaaagagaggctgaagctgatgtttctcaagatttgtttgatcaatttaatttgtttgctcaatattctgctgcagcttattgtgctaaaaataatagggctcctgctggtgctattgttacttgtagagcttctatttgtcctgaagttgaaaaagctgatgctacttttttgtattcttttgaagattctggtgttggtgatgttactggttttttggctttggataatactaatagattgattgttttgtcttttagaggatctaggtcaattgaaaactggattggtaatttgaactatgaattgaaaggtattgatgatatttgttctggttgtaaaggtcatgctggttttacttcttcttggaggtctgttgctaatactttgactcaacaagttcaaaatgctgttagagaacatcctgattatagagttgtttttactggtcattctttgggtggtgctttggctactgttgctggtgcttctttgagaggtaataaatatgatattgatgttttttcttatggtgctccaagagttggtaatagagcttttgctgaatttttgactgctcaaactggtggtactttgtatagaattactcatactaatgatattgttccaagattgccaccaagagaatttggttattctcattcttctcctgaatattggattacttctggtactttggttcctgttagaaggagagatattgttaaagttgaaggtattgattctactgatggtaataatcaaccaaatactccatctattactgctcatttttggtattttggttctattggtacttgtttgtaa

SEQ ID NO: 12 - DNA, 738 bp, synthetic construct
  source 1..738: mol_type = other DNA
tggtcagctgaggacaagcataaggaaggtgtgaatagtcacttatggatcgtgaaccgtgccattgatataatgtctaggaatacaactctggttaagcaagatagagttgctcaattgaatgaatggcgtacagagctagagaatggcatctacgctgctgatcatgaaaacccctattacgatgacagtaccttcgcttctcacttttacgatccagacaacggaaagacatatatcccattcgccaagcaagctaaggagactggagctaagtacttcaagttggctggagagtcatacaagaataaagacatgaagcaggccttcttttatcttgggttgtcattgcattatttgggcgatgtcaaccaacctatgcatgccgcatcctttacggacctgtcctatccacagggttttcactccaagtacgagaactttgtcgatactattaaagacaactacaaagttaccgatgggaacggatattggaattggaaaggcaccaaccctgaagaatggattcacggtgcagcagtagttgcaaaacaggactactctggaattgtcaatgacaataccaaagattggtttgtgaaagccgcagtctcccaggaatatgcagataaatggagagctgaagttacacctatgactggtaaacgactaatggatgcccaaagagttactgctggttacattcaattatggttcgacacttacggtgacaggtaa